European Patent Specification EP 3 793 587 B1, published July 2, 2025. Title: Starting dose of PTH conjugates. Applicant: Ascendis Pharma Bone Diseases A/S. The sequence listing filed with the application follows.

SEQUENCE LISTING (121 sequences)

SEQ ID NO: 1 - protein, 84 aa, Homo sapiens
SVSEIQLMHNLGKHLNSMERVEWLRKKLQDVHNFVALGAPLAPRDAGSQRPRKKEDNVLVESHEKSLGEADKADVNVLTKAKSQ

SEQ ID NO: 2 - protein, 83 aa, Artificial Sequence
  Human PTH 1-83
SVSEIQLMHNLGKHLNSMERVEWLRKKLQDVHNFVALGAPLAPRDAGSQRPRKKEDNVLVESHEKSLGEADKADVNVLTKAKS

SEQ ID NO: 3 - protein, 82 aa, Artificial Sequence
  human PTH 1-82
SVSEIQLMHNLGKHLNSMERVEWLRKKLQDVHNFVALGAPLAPRDAGSQRPRKKEDNVLVESHEKSLGEADKADVNVLTKAK

SEQ ID NO: 4 - protein, 81 aa, Artificial Sequence
  human PTH 1-81
SVSEIQLMHNLGKHLNSMERVEWLRKKLQDVHNFVALGAPLAPRDAGSQRPRKKEDNVLVESHEKSLGEADKADVNVLTKA

SEQ ID NO: 5 - protein, 80 aa, Artificial Sequence
  human PTH 1-80
SVSEIQLMHNLGKHLNSMERVEWLRKKLQDVHNFVALGAPLAPRDAGSQRPRKKEDNVLVESHEKSLGEADKADVNVLTK

SEQ ID NO: 6 - protein, 79 aa, Artificial Sequence
  human PTH 1-79
SVSEIQLMHNLGKHLNSMERVEWLRKKLQDVHNFVALGAPLAPRDAGSQRPRKKEDNVLVESHEKSLGEADKADVNVLT

SEQ ID NO: 7 - protein, 78 aa, Artificial Sequence
  human PTH 1-78
SVSEIQLMHNLGKHLNSMERVEWLRKKLQDVHNFVALGAPLAPRDAGSQRPRKKEDNVLVESHEKSLGEADKADVNVL

SEQ ID NO: 8 - protein, 77 aa, Artificial Sequence
  human PTH 1-77
SVSEIQLMHNLGKHLNSMERVEWLRKKLQDVHNFVALGAPLAPRDAGSQRPRKKEDNVLVESHEKSLGEADKADVNV

SEQ ID NO: 9 - protein, 76 aa, Artificial Sequence
  human PTH 1-76
SVSEIQLMHNLGKHLNSMERVEWLRKKLQDVHNFVALGAPLAPRDAGSQRPRKKEDNVLVESHEKSLGEADKADVN

SEQ ID NO: 10 - protein, 75 aa, Artificial Sequence
  human PTH 1-75
SVSEIQLMHNLGKHLNSMERVEWLRKKLQDVHNFVALGAPLAPRDAGSQRPRKKEDNVLVESHEKSLGEADKADV

SEQ ID NO: 11 - protein, 74 aa, Artificial Sequence
  human PTH 1-74
SVSEIQLMHNLGKHLNSMERVEWLRKKLQDVHNFVALGAPLAPRDAGSQRPRKKEDNVLVESHEKSLGEADKAD

SEQ ID NO: 12 - protein, 73 aa, Artificial Sequence
  human PTH 1-73
SVSEIQLMHNLGKHLNSMERVEWLRKKLQDVHNFVALGAPLAPRDAGSQRPRKKEDNVLVESHEKSLGEADKA

SEQ ID NO: 13 - protein, 72 aa, Artificial Sequence
  human PTH 1-72
SVSEIQLMHNLGKHLNSMERVEWLRKKLQDVHNFVALGAPLAPRDAGSQRPRKKEDNVLVESHEKSLGEADK

SEQ ID NO: 14 - protein, 71 aa, Artificial Sequence
  human PTH 1-71
SVSEIQLMHNLGKHLNSMERVEWLRKKLQDVHNFVALGAPLAPRDAGSQRPRKKEDNVLVESHEKSLGEAD

SEQ ID NO: 15 - protein, 70 aa, Artificial Sequence
  human PTH 1-70
SVSEIQLMHNLGKHLNSMERVEWLRKKLQDVHNFVALGAPLAPRDAGSQRPRKKEDNVLVESHEKSLGEA

SEQ ID NO: 16 - protein, 69 aa, Artificial Sequence
  human PTH 1-69
SVSEIQLMHNLGKHLNSMERVEWLRKKLQDVHNFVALGAPLAPRDAGSQRPRKKEDNVLVESHEKSLGE

SEQ ID NO: 17 - protein, 68 aa, Artificial Sequence
  human PTH 1-68
SVSEIQLMHNLGKHLNSMERVEWLRKKLQDVHNFVALGAPLAPRDAGSQRPRKKEDNVLVESHEKSLG

SEQ ID NO: 18 - protein, 67 aa, Artificial Sequence
  human PTH 1-67
SVSEIQLMHNLGKHLNSMERVEWLRKKLQDVHNFVALGAPLAPRDAGSQRPRKKEDNVLVESHEKSL

SEQ ID NO: 19 - protein, 66 aa, Artificial Sequence
  human PTH 1-66
SVSEIQLMHNLGKHLNSMERVEWLRKKLQDVHNFVALGAPLAPRDAGSQRPRKKEDNVLVESHEKS

SEQ ID NO: 20 - protein, 65 aa, Artificial Sequence
  human PTH 1-65
SVSEIQLMHNLGKHLNSMERVEWLRKKLQDVHNFVALGAPLAPRDAGSQRPRKKEDNVLVESHEK

SEQ ID NO: 21 - protein, 64 aa, Artificial Sequence
  human PTH 1-64
SVSEIQLMHNLGKHLNSMERVEWLRKKLQDVHNFVALGAPLAPRDAGSQRPRKKEDNVLVESHE

SEQ ID NO: 22 - protein, 63 aa, Artificial Sequence
  human PTH 1-63
SVSEIQLMHNLGKHLNSMERVEWLRKKLQDVHNFVALGAPLAPRDAGSQRPRKKEDNVLVESH

SEQ ID NO: 23 - protein, 62 aa, Artificial Sequence
  human PTH 1-62
SVSEIQLMHNLGKHLNSMERVEWLRKKLQDVHNFVALGAPLAPRDAGSQRPRKKEDNVLVES

SEQ ID NO: 24 - protein, 61 aa, Artificial Sequence
  human PTH 1-61
SVSEIQLMHNLGKHLNSMERVEWLRKKLQDVHNFVALGAPLAPRDAGSQRPRKKEDNVLVE

SEQ ID NO: 25 - protein, 60 aa, Artificial Sequence
  human PTH 1-60
SVSEIQLMHNLGKHLNSMERVEWLRKKLQDVHNFVALGAPLAPRDAGSQRPRKKEDNVLV

SEQ ID NO: 26 - protein, 59 aa, Artificial Sequence
  human PTH 1-59
SVSEIQLMHNLGKHLNSMERVEWLRKKLQDVHNFVALGAPLAPRDAGSQRPRKKEDNVL

SEQ ID NO: 27 - protein, 58 aa, Artificial Sequence
  human PTH 1-58
SVSEIQLMHNLGKHLNSMERVEWLRKKLQDVHNFVALGAPLAPRDAGSQRPRKKEDNV

SEQ ID NO: 28 - protein, 57 aa, Artificial Sequence
  human PTH 1-57
SVSEIQLMHNLGKHLNSMERVEWLRKKLQDVHNFVALGAPLAPRDAGSQRPRKKEDN

SEQ ID NO: 29 - protein, 56 aa, Artificial Sequence
  human PTH 1-56
SVSEIQLMHNLGKHLNSMERVEWLRKKLQDVHNFVALGAPLAPRDAGSQRPRKKED

SEQ ID NO: 30 - protein, 55 aa, Artificial Sequence
  human PTH 1-55
SVSEIQLMHNLGKHLNSMERVEWLRKKLQDVHNFVALGAPLAPRDAGSQRPRKKE

SEQ ID NO: 31 - protein, 54 aa, Artificial Sequence
  human PTH 1-54
SVSEIQLMHNLGKHLNSMERVEWLRKKLQDVHNFVALGAPLAPRDAGSQRPRKK

SEQ ID NO: 32 - protein, 53 aa, Artificial Sequence
  human PTH 1-53
SVSEIQLMHNLGKHLNSMERVEWLRKKLQDVHNFVALGAPLAPRDAGSQRPRK

SEQ ID NO: 33 - protein, 52 aa, Artificial Sequence
  human PTH 1-52
SVSEIQLMHNLGKHLNSMERVEWLRKKLQDVHNFVALGAPLAPRDAGSQRPR

SEQ ID NO: 34 - protein, 51 aa, Artificial Sequence
  human PTH 1-51
SVSEIQLMHNLGKHLNSMERVEWLRKKLQDVHNFVALGAPLAPRDAGSQRP

SEQ ID NO: 35 - protein, 50 aa, Artificial Sequence
  human PTH 1-50
SVSEIQLMHNLGKHLNSMERVEWLRKKLQDVHNFVALGAPLAPRDAGSQR

SEQ ID NO: 36 - protein, 49 aa, Artificial Sequence
  human PTH 1-49
SVSEIQLMHNLGKHLNSMERVEWLRKKLQDVHNFVALGAPLAPRDAGSQ

SEQ ID NO: 37 - protein, 48 aa, Artificial Sequence
  human PTH 1-48
SVSEIQLMHNLGKHLNSMERVEWLRKKLQDVHNFVALGAPLAPRDAGS

SEQ ID NO: 38 - protein, 47 aa, Artificial Sequence
  human PTH 1-47
SVSEIQLMHNLGKHLNSMERVEWLRKKLQDVHNFVALGAPLAPRDAG

SEQ ID NO: 39 - protein, 46 aa, Artificial Sequence
  human PTH 1-46
SVSEIQLMHNLGKHLNSMERVEWLRKKLQDVHNFVALGAPLAPRDA

SEQ ID NO: 40 - protein, 45 aa, Artificial Sequence
  human PTH 1-45
SVSEIQLMHNLGKHLNSMERVEWLRKKLQDVHNFVALGAPLAPRD

SEQ ID NO: 41 - protein, 44 aa, Artificial Sequence
  human PTH 1-44
SVSEIQLMHNLGKHLNSMERVEWLRKKLQDVHNFVALGAPLAPR

SEQ ID NO: 42 - protein, 43 aa, Artificial Sequence
  human PTH 1-43
SVSEIQLMHNLGKHLNSMERVEWLRKKLQDVHNFVALGAPLAP

SEQ ID NO: 43 - protein, 42 aa, Artificial Sequence
  human PTH 1-42
SVSEIQLMHNLGKHLNSMERVEWLRKKLQDVHNFVALGAPLA

SEQ ID NO: 44 - protein, 41 aa, Artificial Sequence
  human PTH-41
SVSEIQLMHNLGKHLNSMERVEWLRKKLQDVHNFVALGAPL

SEQ ID NO: 45 - protein, 40 aa, Artificial Sequence
  human PTH 1-40
SVSEIQLMHNLGKHLNSMERVEWLRKKLQDVHNFVALGAP

SEQ ID NO: 46 - protein, 39 aa, Artificial Sequence
  human PTH 1-39
SVSEIQLMHNLGKHLNSMERVEWLRKKLQDVHNFVALGA

SEQ ID NO: 47 - protein, 38 aa, Artificial Sequence
  human PTH 1-38
SVSEIQLMHNLGKHLNSMERVEWLRKKLQDVHNFVALG

SEQ ID NO: 48 - protein, 37 aa, Artificial Sequence
  human PTH 1-37
SVSEIQLMHNLGKHLNSMERVEWLRKKLQDVHNFVAL

SEQ ID NO: 49 - protein, 36 aa, Artificial Sequence
  human PTH 1-36
SVSEIQLMHNLGKHLNSMERVEWLRKKLQDVHNFVA

SEQ ID NO: 50 - protein, 35 aa, Artificial Sequence
  human PTH 1-35
SVSEIQLMHNLGKHLNSMERVEWLRKKLQDVHNFV

SEQ ID NO: 51 - protein, 34 aa, Artificial Sequence
  human PTH 1-34
SVSEIQLMHNLGKHLNSMERVEWLRKKLQDVHNF

SEQ ID NO: 52 - protein, 33 aa, Artificial Sequence
  human PTH 1-33
SVSEIQLMHNLGKHLNSMERVEWLRKKLQDVHN

SEQ ID NO: 53 - protein, 32 aa, Artificial Sequence
  human PTH 1-32
SVSEIQLMHNLGKHLNSMERVEWLRKKLQDVH

SEQ ID NO: 54 - protein, 31 aa, Artificial Sequence
  human PTH 1-31
SVSEIQLMHNLGKHLNSMERVEWLRKKLQDV

SEQ ID NO: 55 - protein, 30 aa, Artificial Sequence
  human PTH 1-30
SVSEIQLMHNLGKHLNSMERVEWLRKKLQD

SEQ ID NO: 56 - protein, 29 aa, Artificial Sequence
  human PTH 1-29
SVSEIQLMHNLGKHLNSMERVEWLRKKLQ

SEQ ID NO: 57 - protein, 28 aa, Artificial Sequence
  human PTH 1-28
SVSEIQLMHNLGKHLNSMERVEWLRKKL

SEQ ID NO: 58 - protein, 27 aa, Artificial Sequence
  human PTH 1-27
SVSEIQLMHNLGKHLNSMERVEWLRKK

SEQ ID NO: 59 - protein, 26 aa, Artificial Sequence
  human PTH 1-26
SVSEIQLMHNLGKHLNSMERVEWLRK

SEQ ID NO: 60 - protein, 25 aa, Artificial Sequence
  human PTH 1-25
SVSEIQLMHNLGKHLNSMERVEWLR

SEQ ID NO: 61 - protein, 84 aa, Artificial Sequence; identical to SEQ ID NO: 1
  amidated human PTH 1-84
  MOD_RES (84)..(84): AMIDATION

SEQ ID NO: 62 - protein, 83 aa, Artificial Sequence; identical to SEQ ID NO: 2
  amidated human PTH 1-83
  MOD_RES (83)..(83): AMIDATION

SEQ ID NO: 63 - protein, 82 aa, Artificial Sequence; identical to SEQ ID NO: 3
  amidated human PTH 1-82
  MOD_RES (82)..(82): AMIDATION

SEQ ID NO: 64 - protein, 81 aa, Artificial Sequence; identical to SEQ ID NO: 4
  amidated human PTH 1-81
  MOD_RES (81)..(81): AMIDATION

SEQ ID NO: 65 - protein, 80 aa, Artificial Sequence; identical to SEQ ID NO: 5
  amidated human PTH 1-80
  MOD_RES (80)..(80): AMIDATION

SEQ ID NO: 66 - protein, 79 aa, Artificial Sequence; identical to SEQ ID NO: 6
  amidated human PTH 1-79
  MOD_RES (79)..(79): AMIDATION

SEQ ID NO: 67 - protein, 78 aa, Artificial Sequence; identical to SEQ ID NO: 7
  amidated human PTH 1-78
  MOD_RES (78)..(78): AMIDATION

SEQ ID NO: 68 - protein, 77 aa, Artificial Sequence; identical to SEQ ID NO: 8
  amidated human PTH 1-77
  MOD_RES (77)..(77): AMIDATION

SEQ ID NO: 69 - protein, 76 aa, Artificial Sequence; identical to SEQ ID NO: 9
  amidated human PTH 1-76
  MOD_RES (76)..(76): AMIDATION

SEQ ID NO: 70 - protein, 75 aa, Artificial Sequence; identical to SEQ ID NO: 10
  amidated human PTH 1-75
  MOD_RES (75)..(75): AMIDATION

SEQ ID NO: 71 - protein, 74 aa, Artificial Sequence; identical to SEQ ID NO: 11
  amidated human PTH 1-74
  MOD_RES (74)..(74): AMIDATION

SEQ ID NO: 72 - protein, 73 aa, Artificial Sequence; identical to SEQ ID NO: 12
  amidated human PTH 1-73
  MOD_RES (73)..(73): AMIDATION

SEQ ID NO: 73 - protein, 72 aa, Artificial Sequence; identical to SEQ ID NO: 13
  amidated human PTH 1-72
  MOD_RES (72)..(72): AMIDATION

SEQ ID NO: 74 - protein, 71 aa, Artificial Sequence; identical to SEQ ID NO: 14
  amidated human PTH 1-71
  MOD_RES (71)..(71): AMIDATION

SEQ ID NO: 75 - protein, 70 aa, Artificial Sequence; identical to SEQ ID NO: 15
  amidated human PTH 1-70
  MOD_RES (70)..(70): AMIDATION

SEQ ID NO: 76 - protein, 69 aa, Artificial Sequence; identical to SEQ ID NO: 16
  amidated human PTH 1-69
  MOD_RES (69)..(69): AMIDATION

SEQ ID NO: 77 - protein, 68 aa, Artificial Sequence; identical to SEQ ID NO: 17
  amidated human PTH 1-68
  MOD_RES (68)..(68): AMIDATION

SEQ ID NO: 78 - protein, 67 aa, Artificial Sequence; identical to SEQ ID NO: 18
  amidated human PTH 1-67
  MOD_RES (67)..(67): AMIDATION

SEQ ID NO: 79 - protein, 66 aa, Artificial Sequence; identical to SEQ ID NO: 19
  amidated human PTH 1-66
  MOD_RES (66)..(66): AMIDATION

SEQ ID NO: 80 - protein, 65 aa, Artificial Sequence; identical to SEQ ID NO: 20
  amidated human PTH 1-65
  MOD_RES (65)..(65): AMIDATION

SEQ ID NO: 81 - protein, 64 aa, Artificial Sequence; identical to SEQ ID NO: 21
  amidated human PTH 1-64
  MOD_RES (64)..(64): AMIDATION

SEQ ID NO: 82 - protein, 63 aa, Artificial Sequence; identical to SEQ ID NO: 22
  amidated human PTH 1-63
  MOD_RES (63)..(63): AMIDATION

SEQ ID NO: 83 - protein, 62 aa, Artificial Sequence; identical to SEQ ID NO: 23
  amidated human PTH 1-62
  MOD_RES (62)..(62): AMIDATION

SEQ ID NO: 84 - protein, 61 aa, Artificial Sequence; identical to SEQ ID NO: 24
  amidated human PTH 1-61
  MOD_RES (61)..(61): AMIDATION

SEQ ID NO: 85 - protein, 60 aa, Artificial Sequence; identical to SEQ ID NO: 25
  amidated human PTH 1-60
  MOD_RES (60)..(60): ACETYLATION

SEQ ID NO: 86 - protein, 59 aa, Artificial Sequence; identical to SEQ ID NO: 26
  amidated human PTH 1-59
  MOD_RES (59)..(59): AMIDATION

SEQ ID NO: 87 - protein, 58 aa, Artificial Sequence; identical to SEQ ID NO: 27
  amidated human PTH 1-58
  MOD_RES (58)..(58): AMIDATION

SEQ ID NO: 88 - protein, 57 aa, Artificial Sequence; identical to SEQ ID NO: 28
  amidated human PTH 1-57
  MOD_RES (57)..(57): AMIDATION

SEQ ID NO: 89 - protein, 56 aa, Artificial Sequence; identical to SEQ ID NO: 29
  amidated human PTH 1-56
  MOD_RES (56)..(56): AMIDATION

SEQ ID NO: 90 - protein, 55 aa, Artificial Sequence; identical to SEQ ID NO: 30
  amidated human PTH 1-55
  MOD_RES (55)..(55): AMIDATION

SEQ ID NO: 91 - protein, 54 aa, Artificial Sequence; identical to SEQ ID NO: 31
  amidated human PTH 1-54
  MOD_RES (54)..(54): AMIDATION

SEQ ID NO: 92 - protein, 53 aa, Artificial Sequence; identical to SEQ ID NO: 32
  amidated human PTH 1-53
  MOD_RES (53)..(53): AMIDATION

SEQ ID NO: 93 - protein, 52 aa, Artificial Sequence; identical to SEQ ID NO: 33
  amidated human PTH 1-52
  MOD_RES (52)..(52): AMIDATION

SEQ ID NO: 94 - protein, 51 aa, Artificial Sequence; identical to SEQ ID NO: 34
  amidated human PTH 1-51
  MOD_RES (51)..(51): AMIDATION

SEQ ID NO: 95 - protein, 50 aa, Artificial Sequence; identical to SEQ ID NO: 35
  amidated human PTH 1-50
  MOD_RES (50)..(50): AMIDATION

SEQ ID NO: 96 - protein, 49 aa, Artificial Sequence; identical to SEQ ID NO: 36
  amidated human PTH 1-49
  MOD_RES (49)..(49): AMIDATION

SEQ ID NO: 97 - protein, 48 aa, Artificial Sequence; identical to SEQ ID NO: 37
  amidated human PTH 1-48
  MOD_RES (48)..(48): AMIDATION

SEQ ID NO: 98 - protein, 47 aa, Artificial Sequence; identical to SEQ ID NO: 38
  amidated human PTH 1-47
  MOD_RES (47)..(47): AMIDATION

SEQ ID NO: 99 - protein, 46 aa, Artificial Sequence; identical to SEQ ID NO: 39
  amidated human PTH 1-46
  MOD_RES (46)..(46): AMIDATION

SEQ ID NO: 100 - protein, 45 aa, Artificial Sequence; identical to SEQ ID NO: 40
  amidated human PTH 1-45
  MOD_RES (45)..(45): AMIDATION

SEQ ID NO: 101 - protein, 44 aa, Artificial Sequence; identical to SEQ ID NO: 41
  amidated human PTH 1-44
  MOD_RES (44)..(44): AMIDATION

SEQ ID NO: 102 - protein, 43 aa, Artificial Sequence; identical to SEQ ID NO: 42
  amidated human PTH 1-43
  MOD_RES (43)..(43): AMIDATION

SEQ ID NO: 103 - protein, 42 aa, Artificial Sequence; identical to SEQ ID NO: 43
  amidated human PTH 1-42
  MOD_RES (42)..(42): AMIDATION

SEQ ID NO: 104 - protein, 41 aa, Artificial Sequence; identical to SEQ ID NO: 44
  amidated human PTH 1-41
  MOD_RES (41)..(41): AMIDATION

SEQ ID NO: 105 - protein, 40 aa, Artificial Sequence; identical to SEQ ID NO: 45
  amidated human PTH 1-40
  MOD_RES (40)..(40): AMIDATION

SEQ ID NO: 106 - protein, 39 aa, Artificial Sequence; identical to SEQ ID NO: 46
  amidated human PTH 1-39
  MOD_RES (39)..(39): AMIDATION

SEQ ID NO: 107 - protein, 38 aa, Artificial Sequence; identical to SEQ ID NO: 47
  amidated human PTH 1-38
  MOD_RES (38)..(38): AMIDATION

SEQ ID NO: 108 - protein, 37 aa, Artificial Sequence; identical to SEQ ID NO: 48
  amidated human PTH 1-37
  MOD_RES (37)..(37): AMIDATION

SEQ ID NO: 109 - protein, 36 aa, Artificial Sequence; identical to SEQ ID NO: 49
  amidated human PTH 1-36
  MOD_RES (36)..(36): AMIDATION

SEQ ID NO: 110 - protein, 35 aa, Artificial Sequence; identical to SEQ ID NO: 50
  amidated human PTH 1-35
  MOD_RES (35)..(35): AMIDATION

SEQ ID NO: 111 - protein, 34 aa, Artificial Sequence; identical to SEQ ID NO: 51
  amidated human PTH 1-34
  MOD_RES (34)..(34): AMIDATION

SEQ ID NO: 112 - protein, 33 aa, Artificial Sequence; identical to SEQ ID NO: 52
  amidated human PTH 1-33
  MOD_RES (33)..(33): AMIDATION

SEQ ID NO: 113 - protein, 32 aa, Artificial Sequence; identical to SEQ ID NO: 53
  amidated human PTH 1-32
  MOD_RES (32)..(32): AMIDATION

SEQ ID NO: 114 - protein, 31 aa, Artificial Sequence; identical to SEQ ID NO: 54
  amidated human PTH 1-31
  MOD_RES (31)..(31): AMIDATION

SEQ ID NO: 115 - protein, 30 aa, Artificial Sequence; identical to SEQ ID NO: 55
  amidated human PTH 1-30
  MOD_RES (30)..(30): AMIDATION

SEQ ID NO: 116 - protein, 29 aa, Artificial Sequence
  amidated human PTH 1-29
  MOD_RES (29)..(29): AMIDATION
SVSEIQLMHNLGKHLNSMERVEWLRKKLQ

SEQ ID NO: 117 - protein, 28 aa, Artificial Sequence
  amidated human PTH 1-28
  MOD_RES (28)..(28): AMIDATION
SVSEIQLMHNLGKHLNSMERVEWLRKKL

SEQ ID NO: 118 - protein, 27 aa, Artificial Sequence
  amidated human PTH 1-27
  MOD_RES (27)..(27): AMIDATION
SVSEIQLMHNLGKHLNSMERVEWLRKK

SEQ ID NO: 119 - protein, 26 aa, Artificial Sequence
  amidated human PTH 1-26
  MOD_RES (26)..(26): AMIDATION
SVSEIQLMHNLGKHLNSMERVEWLRK

SEQ ID NO: 120 - protein, 25 aa, Artificial Sequence
  amidated human PTH 1-25
  MOD_RES (25)..(25): AMIDATION
SVSEIQLMHNLGKHLNSMERVEWLR

SEQ ID NO: 121 - protein, 141 aa, Homo sapiens
AVSEHQLLHDKGKSIQDLRRRFFLHHLIAEIHTAEIRATSEVSPNSKPSPNTKNHPVRFGSDDEGRYLTQETNKVETYKEQPLKTPGKKKKGKPGKRKEQEKKKRRTRSAWLDSGVTGSGLEGDHLSDTSTTSLELDSRRH